European Patent Application EP 4 748 853 A1, published May 27, 2026. Title: 一种角蛋白CF8、制法和其药物组合物与用途. Applicant: 中国医学科学院药物研究所. The sequence listing filed with the application follows.

SEQUENCE LISTING (2 sequences)

SEQ ID NO: 1 - protein, 459 aa, unidentified
MTTCSRQFTSSSSLKGSCGIGGGSSRISSILGGGSYQAPSAYGGGLSVSSRYSSGGACGLGGGYGGGFSSSSSFGGALGSGFGGGYGGGLGAGFGAGFGGGFIGGDGGLISGNEKITMQNLNDRLASYLDKVRALEEANAELEVKIRDWYLKQRPTEPKDYSPYFRTIEDLRNKIITATIENAQPILQIDNARLAADDFRTKYEHELALRQSVEADINGLRRVLDELTLARTDLEMQIESLKEELAYLRKNHQEEMLALRSQTGGDVNVEMDAAPSVDLSRILNEMRDQYEQIAEKNRRDAEAWFLRKTEELNKEVASNSELVQTSRSEVTELRRVLQGLEIELQSQLSLKASLENSLEETKGRYCLQLSQIQGLISSVEEQLAQLRCEMEQQSQEYQILLDVKTRLEQEIATYRRLLEGEDAHLSSQHTSSQSYSSRDVISSSSSTSSSRQTRPIHKE

SEQ ID NO: 2 - DNA, 1377 bp, unidentified
  source 1..1377: mol_type = other DNA
atgaccacctgcagccgccagtttaccagcagctcaagcctgaaaggcagctgcggtattggcggtggtagcagccgtattagcagcattctgggtggtggcagctatcaggcgccgagcgcgtatggcggtggtttaagcgttagcagccgctatagcagcggcggcgcgtgtggtttaggtggtggttatggtggtggttttagcagcagcagcagctttggtggtgcgttaggcagcggctttggcggtggttatggcggcggtttaggcgcgggctttggtgcgggttttggcggcggttttattggcggtgatggcggtttaattagcggcaatgaaaaaattaccatgcagaacctgaacgaccgcctggcgagctatctggataaagtgcgcgcgctggaagaagcgaacgcggaattagaagtgaaaattcgcgattggtatctgaagcagcgcccgaccgaaccgaaagattatagcccgtattttcgcaccattgaggatctgcgcaacaaaattattaccgcgaccattgaaaacgcgcagccgattctgcagattgataacgcgcgcctggcggcggatgattttcgcaccaaatatgaacatgaactggcgctgcgccagagcgtggaagcggatattaatggcctgcgccgcgttttagatgaactgaccttagcgcgtaccgatctggaaatgcagattgaaagcctgaaagaagaactggcgtatctgcgcaaaaaccatcaggaagaaatgctggcgctgcgcagccagaccggtggtgatgttaatgtggaaatggatgcggcgccgagcgtggatttaagccgtattctgaatgaaatgcgcgatcagtatgaacagattgcggaaaaaaaccgccgcgatgcggaagcgtggtttctgcgtaaaaccgaagaactgaacaaagaggtggcgagcaacagcgaactggtgcagactagccgtagcgaagttaccgaattacgccgtgtgctgcagggcctggaaattgaactgcagagccagctgagcctgaaagcgagcttagaaaacagcctggaagaaaccaaaggccgctattgcctgcagctgagccagattcagggcctgattagcagcgtggaagaacagctggcgcagctgcgttgtgaaatggaacagcaaagccaggaatatcagattctgctggatgtgaaaacccgcctggaacaggaaattgcgacctatcgccgcctgctggaaggcgaagatgcgcatttaagcagccagcataccagcagccaaagctatagcagccgcgatgtgattagcagcagcagcagcaccagcagcagccgccaaactcgtcctattcataaagaa